European Patent Specification EP 4 028 549 B1, published June 11, 2025. Title: Method for the production of rAAV and method for the in vitro generation of genetically engineered, linear, single-stranded nucleic acid fragments containing ITR sequences flanking a gene of interest. Applicant: Universitaet Bielefeld. The sequence listing filed with the application follows.

SEQUENCE LISTING (7 sequences)

SEQ ID NO: 1 - DNA, 4792 bp, artificial
  genetically engineered plasmid of the example
  rep_origin (1)..(422): in combination with rep_origin 4595 to 4792
  misc_feature (469)..(609): ITR
  promoter (659)..(1312)
  CDS (1319)..(2014): mKate2
  polyA_site (2023)..(2501): complement
  polyA_signal (2105)..(2110)
  misc_feature (2534)..(2663): ITR complement
  rep_origin (2755)..(3061)
  promoter (3510)..(3538)
  CDS (3580)..(4440): AmpR
  rep_origin (4595)..(4792): in combination with rep_origin of 1 to 422
agaactctgtagcaccgcctacatacctcgctctgctaatcctgttaccagtggctgctgccagtggcgataagtcgtgtcttaccgggttggactcaagacgatagttaccggataaggcgcagcggtcgggctgaacggggggttcgtgcacacagcccagcttggagcgaacgacctacaccgaactgagatacctacagcgtgagctatgagaaagcgccacgcttcccgaagggagaaaggcggacaggtatccggtaagcggcagggtcggaacaggagagcgcacgagggagcttccagggggaaacgcctggtatctttatagtcctgtcgggtttcgccacctctgacttgagcgtcgatttttgtgatgctcgtcaggggggcggagcctatggaaaaacgccagcaacgcggcctttttacggttcctggccttttgctggccttttgctcacatgtcctgcaggcagctgcgcgctcgctcgctcactgaggccgcccgggcaaagcccgggcgtcgggcgacctttggtcgcccggcctcagtgagcgagcgagcgcgcagagagggagtggccaactccatcactaggggttcctgcggccgcctatcgagaccggcgccgcgaattcgcggccgcttctagagcgatgtacgggccagatatacgcgttgacattgattattgcctagttattaatagtaatcaattacggggtcattagttcatagcccatatatggagttccgcgttacataacttacggtaaatggcccgcctggctgaccgcccaacgacccccgcccattgacgtcaataatgacgtatgttcccatagtaacgccaatagggactttccattgacgtcaatgggtggagtatttacggtaaactgcccacttggcagtacatcaagtgtatcatatgccaagtacgccccctattgacgtcaatgacggtaaatggcccgcctggcattatgcccagtacatgaccttatgggactttcctacttggcagtacatctacgtattagtcatcgctattaccatggtgatgcggttttggcagtacatcaatgggcgtggatagcggtttgactcacggggatttccaagtctccaccccattgacgtcaatgggagtttgttttggcaccaaaatcaacgggactttccaaaatgtcgtaacaactccgccccattgacgcaaatgggcggtaggcgtgtacggtgggaggtctatataagcagagctctctggctaactagagaacccactgcttactggcttatcgaaattactagatggtgtctgagctgatcaaagaaaacatgcacatgaagctgtacatggaaggcaccgtgaacaaccaccacttcaagtgcacctccgagggcgagggcaagccttatgagggcacccagaccatgcggatcaaggccgtggaaggcggccctctgcctttcgcctttgatatcctggccacctcctttatgtacggctccaagaccttcatcaaccacacccagggcatccccgatttcttcaagcagagcttccccgagggcttcacctgggagagagtgaccacctacgaggacggcggcgtgctgaccgctacccaggatacctctctccaggacggctgcctgatctacaacgtgaagatccggggcgtgaacttcccctccaacggccccgtgatgcagaagaaaaccctgggctgggaggccagcaccgagacactgtatcctgctgacggcggcctggaaggcagagccgatatggccctgaaactcgtgggcggaggccacctgatctgtaacctgaaaaccacctaccggtccaagaagcccgccaagaacctgaagatgcccggcgtgtactacgtggaccggcggctggaacggatcaaagaggccgacaaagaaacctacgtggaacagcacgaggtggccgtggccagatactgcgacctgcctagcaagctgggccacagatactagagacgggtggcatccctgtgacccctccccagtgcctctcctggccctggaagttgccactccagtgcccaccagccttgtcctaataaaattaagttgcatcattttgtctgactaggtgtccttctataatattatggggtggaggggggtggtatggagcaaggggcaagttgggaagacaacctgtagggcctgcggggtctattgggaaccaagctggagtgcagtggcacaatcttggctcactgcaatctccgcctcctgggttcaagcgattctcctgcctcagcctcccgagttgttgggattccaggcatgcatgaccaggctcagctaatttttgtttttttggtagagacggggtttcaccatattggccaggctggtctccaactcctaatctcaggtgatctacccaccttggcctcccaaattgctgggattacaggcgtgaaccactgctcccttccctgtcctttactagtaccggtggtctctggcggcggccgcaggaacccctagtgatggagttggccactccctctctgcgcgctcgctcgctcactgaggccgggcgaccaaaggtcgcccgacgcccgggcggcctcagtgagcgagcgagcgcgcagctgcctgcaggggcgcctgatgcggtattttctccttacgcatctgtgcggtatttcacaccgcatacgtcaaagcaaccatagtacgcgccctgtagcggcgcattaagcgcggcgggtgtggtggttacgcgcagcgtgaccgctacacttgccagcgccctagcgcccgctcctttcgctttcttcccttcctttctcgccacgttcgccggctttccccgtcaagctctaaatcgggggctccctttagggttccgatttagtgctttacggcacctcgaccccaaaaaacttgatttgggtgatggttcacgtagtgggccatcgccctgatagacggtttttcgccctttgacgttggagtccacgttctttaatagtggactcttgttccaaactggaacaacactcaaccctatctcgggctattcttttgatttataagggattttgccgatttcggcctattggttaaaaaatgagctgatttaacaaaaatttaacgcgaattttaacaaaatattaacgtttacaattttatggtgcactctcagtacaatctgctctgatgccgcatagttaagccagccccgacacccgccaacacccgctgacgcgccctgacgggcttgtctgctcccggcatccgcttacagacaagctgtgaccgtctccgggagctgcatgtgtcagaggttttcaccgtcatcaccgaaacgcgcgagacgaaagggcctcgtgatacgcctatttttataggttaatgtcatgataataatggtttcttagacgtcaggtggcacttttcggggaaatgtgcgcggaacccctatttgtttatttttctaaatacattcaaatatgtatccgctcatgagacaataaccctgataaatgcttcaataatattgaaaaaggaagagtatgagtattcaacatttccgtgtcgcccttattcccttttttgcggcattttgccttcctgtttttgctcacccagaaacgctggtgaaagtaaaagatgctgaagatcagttgggtgcacgagtgggttacatcgaactggatctcaacagcggtaagatccttgagagttttcgccccgaagaacgttttccaatgatgagcacttttaaagttctgctatgtggcgcggtattatcccgtattgacgccgggcaagagcaactcggtcgccgcatacactattctcagaatgacttggttgagtactcaccagtcacagaaaagcatcttacggatggcatgacagtaagagaattatgcagtgctgccataaccatgagtgataacactgcggccaacttacttctgacaacgatcggaggaccgaaggagctaaccgcttttttgcacaacatgggggatcatgtaactcgccttgatcgttgggaaccggagctgaatgaagccataccaaacgacgagcgtgacaccacgatgcctgtagcaatggcaacaacgttgcgcaaactattaactggcgaactacttactctagcttcccggcaacaattaatagactggatggaggcggataaagttgcaggaccacttctgcgctcggcccttccggctggctggtttattgctgataaatctggagccggtgagcgtggctcgcgcggtatcattgcagcactggggccagatggtaagccctcccgtatcgtagttatctacacgacggggagtcaggcaactatggatgaacgaaatagacagatcgctgagataggtgcctcactgattaagcattggtaactgtcagaccaagtttactcatatatactttagattgatttaaaacttcatttttaatttaaaaggatctaggtgaagatcctttttgataatctcatgaccaaaatcccttaacgtgagttttcgttccactgagcgtcagaccccgtagaaaagatcaaaggatcttcttgagatcctttttttctgcgcgtaatctgctgcttgcaaacaaaaaaaccaccgctaccagcggtggtttgtttgccggatcaagagctaccaactctttttccgaaggtaactggcttcagcagagcgcagataccaaatactgtccttctagtgtagccgtagttaggccaccacttca

SEQ ID NO: 2 - protein, 232 aa, artificial
  Synthetic Construct
MVSELIKENMHMKLYMEGTVNNHHFKCTSEGEGKPYEGTQTMRIKAVEGGPLPFAFDILATSFMYGSKTFINHTQGIPDFFKQSFPEGFTWERVTTYEDGGVLTATQDTSLQDGCLIYNVKIRGVNFPSNGPVMQKKTLGWEASTETLYPADGGLEGRADMALKLVGGGHLICNLKTTYRSKKPAKNLKMPGVYYVDRRLERIKEADKETYVEQHEVAVARYCDLPSKLGHR

SEQ ID NO: 3 - protein, 286 aa, artificial
  Synthetic Construct
MSIQHFRVALIPFFAAFCLPVFAHPETLVKVKDAEDQLGARVGYIELDLNSGKILESFRPEERFPMMSTFKVLLCGAVLSRIDAGQEQLGRRIHYSQNDLVEYSPVTEKHLTDGMTVRELCSAAITMSDNTAANLLLTTIGGPKELTAFLHNMGDHVTRLDRWEPELNEAIPNDERDTTMPVAMATTLRKLLTGELLTLASRQQLIDWMEADKVAGPLLRSALPAGWFIADKSGAGERGSRGIIAALGPDGKPSRIVVIYTTGSQATMDERNRQIAEIGASLIKHW

SEQ ID NO: 4 - DNA, 11 bp, artificial
  deletion ITR
tttgcccgggc

SEQ ID NO: 5 - DNA, 18 bp, artificial
  primer
ggcggagttgttacgaca

SEQ ID NO: 6 - DNA, 19 bp, artificial
  primer
gggactttcctacttggca

SEQ ID NO: 7 - DNA, 6455 bp, artificial
  plasmid prepcap
  gene (51)..(1982): Rep gene
  gene (1933)..(4140): Cap gene
  rep_origin (4696)..(5315): pBR322 origin
  gene (5597)..(6256): CAT marker complement
atccttagctttcgctaaggatgatttctggaattcgcggccgcttctagatggcggggttttacgagattgtgattaaggtccccagcgaccttgacgagcatctgcccggcatttctgacagctttgtgaactgggtggccgagaaggaatgggagttgccgccagattctgacatggatctgaatctgattgagcaggcacccctgaccgtggccgagaagctccagcgcgactttctgacggaatggcgccgtgtgagtaaggccccggaggcccttttctttgtgcaatttgagaagggagagagctacttccacatgcacgtgctcgtggaaaccaccggggtgaaatccatggttttgggacgtttcctgagtcagattcgcgaaaaactgattcagagaatttaccgcgggatcgagccgactttgccaaactggttcgcggtcacaaagaccagaaatggcgccggaggcgggaacaaggtggtggatgagtgctacatccccaattacttgctccccaaaacccagcctgagctccagtgggcgtggactaatatggaacagtatttaagcgcctgtttgaatctcacggagcgtaaacggttggtggcgcagcatctgacgcacgtgtcgcagacgcaggagcagaacaaagagaatcagaatcccaattctgatgcgccggtgatcagatcaaaaacttcagccaggtacatggagctggtcgggtggctcgtggacaaggggattacctcggagaagcagtggattcaggaggaccaggcctcatacatctccttcaatgcggcctccaactcgcggtcccaaatcaaggctgccttggacaatgcgggaaagattatgagcctgactaaaaccgcccccgactacctggtgggccagcagcccgtggaggacatttccagcaatcggatttataaaattttggaactaaacgggtacgatccccaatatgcggcttccgtctttctgggatgggccacgaaaaagttcggcaagaggaacaccatctggctgtttgggcctgcaactaccgggaagaccaacatcgcggaggccatagcccacactgtgcccttctacgggtgcgtaaactggaccaatgagaactttcccttcaacgactgtgtggacaagatggtgatctggtgggaggaggggaagatgaccgccaaggtcgtggagtcggccaaagccattctcggaggaagcaaggtgcgcgtggaccagaaatgcaagtcctcggcccagatagacccgactcccgtgatcgtcacctccaacaccaacatgtgcgccgtgattgacgggaactcaacgaccttcgaacaccagcagccgttgcaagaccggatgttcaaatttgaactcacccgccgtctggatcatgactttgggaaggtcaccaagcaggaagtcaaagactttttccggtgggcaaaggatcacgtggttgaggtggagcatgagttctacgtcaaaaagggtggagccaagaaaagacccgcccccagtgacgcagatataagtgagcccaaacgggtgcgcgagtcagttgcgcagccatcgacgtcagacgcggaagcttcgatcaactacgcagacaggtaccaaaacaaatgttctcgtcacgtgggcatgaatctgatgctgtttccctgtagacaatgcgagagaatgaatcagaactcaaatatctgcttcactcacggacagaaagactgtttagagtgctttcccgtgtcagaatctcaacccgtttctgtcgtcaaaaaggcgtatcagaaactgtgctacattcatcatatcatgggaaaggtgccagacgcttgcactgcctgcgatctggtcaatgtggatttggatgactgcatctttgaacaataaatgatttaaatcaggtatggctgccgatggttatcttccagattggctcgaggacactctctctgaaggaataagacagtggtggaagctcaaacctggcccaccaccaccaaagcccgcagagcggcataaggacgacagcaggggtcttgtgcttcctgggtacaagtacctcggacccttcaacggactcgacaagggagagccggtcaacgaggcagacgccgcggccctcgagcacgacaaagcctacgaccggcagctcgacagcggagacaacccgtacctcaagtacaaccacgccgacgcggagtttcaggagcgccttaaagaagatacgtcttttgggggcaacctcggacgagcagtcttccaggcgaaaaagagggttcttgaacctctgggcctggttgaggaacctgttaagacggctccgggaaaaaagaggccggtagagcactctcctgtggagccagactcctcctcgggaaccggaaaggcgggccagcagcctgcaagaaaaagattgaattttggtcagactggagacgcagactcagtacctgacccccagcctctcggacagccaccagcagccccctctggtctgggaactaatacgatggctacaggcagtggcgcaccaatggcagacaataacgagggcgccgacggagtgggtaattcctcgggaaattggcattgcgattccacatggatgggcgacagagtcatcaccaccagcacccgaacctgggccctgcccacctacaacaaccacctctacaaacaaatttccagccaatcaggagcctcgaacgacaatcactactttggctacagcaccccttgggggtattttgacttcaacagattccactgccacttttcaccacgtgactggcaaagactcatcaacaacaactggggattccgacccaagagactcaacttcaagctctttaacattcaagtcaaagaggtcacgcagaatgacggtacgacgacgattgccaataaccttaccagcacggttcaggtgtttactgactcggagtaccagctcccgtacgtcctcggctcggcgcatcaaggatgcctcccgccgttcccagcagacgtcttcatggtgccacagtatggatacctcaccctgaacaacgggagtcaggcagtaggacgctcttcattttactgcctggagtactttccttctcagatgctgcgtaccggaaacaactttaccttcagctacacttttgaggacgttcctttccacagcagctacgctcacagccagagtctggaccgtctcatgaatcctctcatcgaccaatatttgtattacttgagcagaacaaacactccaagtggtaccaccacgcagagtcgacttcagttttctcaggccggagcgagtgacattcgggaccagtctaggaactggcttcctggaccctgttaccgccagcagcgagtatcaaagacatctgcggataacaacaacagtgaatactcgtggactggagctaccaagtaccacctcaatggcagagactctctggtgaatccgggcccggccatggcaagccacaaggacgatgaagaaaagttttttcctcagagcggggttctcatctttgggaagcaaggctcagagaaaacaaatgtggacattgaaaaggtcatgattacagacgaagaggaaatcaggacaaccaatcccgtggctacggagcagtatggatccgtatctaccaacctccagagaggcaacagacaagcagctacagctgatgtcaacacacaaggcgttcttccaggcatggtctggcaggacagagatgtgtaccttcaggggcccatctgggcaaagattccacacacggacggacattttcacccctctcccctcatgggtggattcggacttaaacaccctcctccacagattctcatcaagaacaccccggtacctgcgaatccttcgaccaccttcagtgcggcaaagtttgcttccttcatcacacagtactccacgggacaggtcagcgtggagatcgagtgggagctccagaaggaaaacagcaaacgctggaatcccgaaattcagtacacttccaactacaacaagtctgttaatgtggactttactgtggacactaatggcgtgtattcagagcctcgccccattggcaccagatacctgactcgtaatctgtaattgcttgttaatcaataaaccgtttaattcgtttcagttgaactttggtctctgcgtatttctttcttatctagtttccatggctacgtagataagtagcatggcgggttaatcattaactactactagagggaggggtggagtcgtgacgtgaattacgtcatagggttagggaggtcctgtattagaggtcacgtgagtgttttgcgacattttgcgacaccatgtggtctcgctgggggggggggcccgagtgagcacgcagggtctccattttgaagcgggaggtttgaactactagtagcggccgctgcagtccggcaaaaaaacgggcaaggtgtcaccaccctgccctttttctttaaaaccgaaaagattacttcgcgttatgcaggcttcctcgctcactgactcgctgcgctcggtcgttcggctgcggcgagcggtatcagctcactcaaaggcggtaatacggttatccacagaatcaggggataacgcaggaaagaacatgtgagcaaaaggccagcaaaaggccaggaaccgtaaaaaggccgcgttgctggcgtttttccataggctccgcccccctgacgagcatcacaaaaatcgacgctcaagtcagaggtggcgaaacccgacaggactataaagataccaggcgtttccccctggaagctccctcgtgcgctctcctgttccgaccctgccgcttaccggatacctgtccgcctttctcccttcgggaagcgtggcgctttctcatagctcacgctgtaggtatctcagttcggtgtaggtcgttcgctccaagctgggctgtgtgcacgaaccccccgttcagcccgaccgctgcgccttatccggtaactatcgtcttgagtccaacccggtaagacacgacttatcgccactggcagcagccactggtaacaggattagcagagcgaggtatgtaggcggtgctacagagttcttgaagtggtggcctaactacggctacactagaaggacagtatttggtatctgcgctctgctgaagccagttaccttcggaaaaagagttggtagctcttgatccggcaaacaaaccaccgctggtagcggtggtttttttgtttgcaagcagcagattacgcgcagaaaaaaaggatctcaagaagatcctttgatcttttctacggggtctgacgctcagtggaacgaaaactcacgttaagggattttggtcatgagattatcaaaaaggatcttcacctagatccttttaaattaaaaatgaagttttaaatcaatctaaagtatatatgagtaaacttggtctgacagctcgaggcttggattctcaccaataaaaaacgcccggcggcaaccgagcgttctgaacaaatccagatggagttctgaggtcattactggatctatcaacaggagtccaagcgagctcgatatcaaattacgccccgccctgccactcatcgcagtactgttgtaattcattaagcattctgccgacatggaagccatcacaaacggcatgatgaacctgaatcgccagcggcatcagcaccttgtcgccttgcgtatagtatttgcccatggtgaaaacgggggcgaagaagttgtccatattggccacgtttaaatcaaaactggtgaaactcacccagggattggctgagacgaaaaacatattctcaataaaccctttagggaaataggccaggttttcaccgtaacacgccacatcttgcgaatatatgtgtagaaactgccggaaatcgtcgtggtattcactccagagcgatgaaaacgtttcagtttgctcatggaaaacggtgtaacaagggtgaacactatcccatatcaccagctcaccgtctttcattgccatacgaaattccggatgagcattcatcaggcgggcaagaatgtgaataaaggccggataaaacttgtgcttatttttctttacggtctttaaaaaggccgtaatatcgagctgaacggtctggttataggtacattgagcaactgactgaaatgcctcaaaatgttctttacgatgccattgggatatatcaacggtggtatatccagtgatttttttctccattttagcttccttagctcctgaaaatctcgataactcaaaaaatacgcccggtagtgatcttatttcattatggtgaaagttggaacctcttacgtgcccgatcaactcgagtgccacttgacgtctaagaaaccattattatcatgacattaacctataaaaataggcgtatcacgaggcagaatttcagataaaaaaa